European Patent Application EP 4 317 453 A1, published February 7, 2024. Title: Anti-drug antibody assay. Applicant: SEKISUI MEDICAL CO., LTD. The sequence listing filed with the application follows.

SEQUENCE LISTING (4 sequences)

SEQ ID NO: 1 - DNA, 22 bp, Artificial Sequence
  capture nucleic acid
tacgttatcagactgatgttga

SEQ ID NO: 2 - DNA, 61 bp, Artificial Sequence
  tracer nucleic acid
tacgttatcagactgatgttgagatataaggagtggataccgatgaaggatataaggagtg

SEQ ID NO: 3 - DNA, 39 bp, Artificial Sequence
  probe
gtcctgattgttgcttcatcggtatccactccttatatc

SEQ ID NO: 4 - DNA, 39 bp, Artificial Sequence
  probe
caacaatcaggacgataccgatgaaggatataaggagtg